European Patent Specification EP 3 356 384 B1, published November 29, 2023. Title: POLYPEPTIDES COMPRISING VINCULIN BINDING SITES FOR THE TREATMENT OF PROLIFERATION AND/OR ADHESION RELATED DISEASES. Applicant: PARIS SCIENCES ET LETTRES - QUARTIER LATIN CENTRE NATIONAL DE LA RECHERCHE SCIENTIFIQUE INSTITUT NATIONAL DE LA SANTÉ ET DE LA RECHERCHE MÉDICALE TRAN VAN NHIEU Guy. The sequence listing filed with the application follows.

SEQUENCE LISTING (79 sequences)

SEQ ID NO: 1 - protein, 633 aa, Shigella flexneri
  IpaA (1-633)
MHNVNNTQAPTFLYKATSPSSTEYSELKSKISDIHSSQTSLKTPASVSEKENFATSFNQKCLDFLFSSSGKEDVLRSIYSNSMNAYAKSEILEFSNVLYSLVHQNGLNFENEKGLQKIVAQYSELIIKDKLSQDSAFGPWSAKNKKLHQLRQNIEHRLALLAQQHTSGEALSLGQKLLNTEVSSFIKNNILAELKLSNETVSSLKLDDLVDAQAKLAFDSLRNQRKNTIDSKGFGIGKLSRDLNTVAVFPELLRKVLNDILEDIKDSHPIQDGLPTPPEDMPDGGPTPGANEKTSQPVIHYHINNDNRTYDNRVFDNRVYDNSYHENPENDAQSPTSQTNDLLSRNGNSLLNPQRALVQKVTSVLPHSISDTVQTFANNSALEKVFNHTPDNSDGIGSDLLTTSSQERSANNSLSRGHRPLNIQNSSTTPPLHPEGVTSSNDNSSDTTKSSASLSHRVASQINKFNSNTDSKVLQTDFLSRNGDTYLTRETIFEASKKVTNSLSNLISLIGTKSGTQERELQEKSKDITKSTTEHRINNKLKVTDANIRNYVTETNADTIDKNHAIYEKAKEVSSALSKVLSKIDDTSAELLTDDISDLKNNNDITAENNNIYKAAKDVTTSLSKVLKNINKD

SEQ ID NO: 2 - protein, 19 aa, Shigella flexneri
  IpaA VBS1
IYKAAKDVTTSLSKVLKNI

SEQ ID NO: 3 - protein, 19 aa, Shigella flexneri
  IpaA VBS2
IYEKAKEVSSALSKVLSKI

SEQ ID NO: 4 - protein, 19 aa, Shigella flexneri
  IpaA VBS3
IFEASKKVTNSLSNLISLI

SEQ ID NO: 5 - protein, 151 aa, Shigella flexneri
  A483 / IpaA (483-633)
GDTYLTRETIFEASKKVTNSLSNLISLIGTKSGTQERELQEKSKDITKSTTEHRINNKLKVTDANIRNYVTETNADTIDKNHAIYEKAKEVSSALSKVLSKIDDTSAELLTDDISDLKNNNDITAENNNIYKAAKDVTTSLSKVLKNINKD

SEQ ID NO: 6 - DNA, 456 bp, Shigella flexneri
  A483 / IpaA (483-633)
ggagacacatatttaacacgggaaacgatatttgaagcttcaaaaaaagtaacaaactccctaagtaatcttatatctctcattggaactaaatcaggaacacaagaacgagagttacaggaaaaatcaaaggacattacaaaatccacaacagaacatagaataaacaacaaattaaaagttacagatgcaaatataagaaactacgtaacagaaaccaacgcagatacaattgataaaaatcatgcgatctatgaaaaggcaaaagaagtatctagcgccctcagcaaggtattgtcaaaaattgacgatacctctgcagaattacttacagatgatatatctgatttaaaaaataacaatgatattacagctgaaaacaataatatatataaagcagcaaaagatgtaaccacttccctatcaaaagtattaaagaatatcaataaggattaa

SEQ ID NO: 7 - DNA, 1902 bp, Shigella flexneri
  IpaA (1-633)
atgcataatgtaaataatactcaagcgccaacattcttatataaggcaacttcaccatcatcaacagaatacagcgagttaaaaagcaaaatatccgatatccatagttcgcaaacttctctaaaaacaccagcatcagtgtctgaaaaagaaaactttgcaacgtcttttaatcagaaatgtcttgattttttattttcttcctcagggaaagaagatgtgttaagaagcatttattccaactcaatgaatgcgtatgccaaaagcgagattctcgaattttcaaatgttttgtactccttagtacatcaaaatggtcttaattttgaaaacgaaaagggacttcaaaaaattgtcgcacagtattcggaactaattataaaagataaattatcccaagattctgcctttggaccatggtcggcaaagaataagaaactccatcaattacgacaaaacattgagcacagacttgcactattagcacaacaacacacatctggtgaagctttatcattgggacaaaaactcctcaatactgaagtatcatcatttatcaagaataatattcttgctgaattaaagttaagtaatgaaactgtttcatctctcaaactagatgatttagttgacgcacaggcaaaacttgcctttgatagtttgcgcaatcaacgtaaaaatactattgatagtaaaggatttggtataggtaaactgtcaagagacttaaatacagtagccgtgtttcctgagctgttgagaaaagtccttaatgatattttagaagatataaaagattcgcatcctatccaagatggcctccctacacctcccgaagatatgccagatggcggaccaacccccggagccaatgagaaaacatcccaacctgtaattcactatcatataaataatgataatagaacttacgataatagagtttttgacaacagagtatatgacaatagctatcacgagaacccagaaaatgatgcacagtctcctacttctcagacaaacgatctattatcccgtaacggaaactcattactaaatccacaaagagcactagttcaaaaagtaacttccgttctaccacactctatatcagatactgtccagacatttgcaaataattcagctttagaaaaggttttcaaccatactccagataattcggatggaataggttcagacctgttaactacgagtagtcaagaaagatctgcaaataactctctttctcggggacacaggcctctgaacatacagaactcttcaaccaccccccctctccacccggaaggagtgacaagcagtaatgataactcatcagatacaactaaaagtagcgcttctctttctcatagagtagcttcgcaaatcaataaattcaactcaaacactgattcaaaagtacttcagactgattttttatcaagaaatggagacacatatttaacacgggaaacgatatttgaagcttcaaaaaaagtaacaaactccctaagtaatcttatatctctcattggaactaaatcaggaacacaagaacgagagttacaggaaaaatcaaaggacattacaaaatccacaacagaacatagaataaacaacaaattaaaagttacagatgcaaatataagaaactacgtaacagaaaccaacgcagatacaattgataaaaatcatgcgatctatgaaaaggcaaaagaagtatctagcgccctcagcaaggtattgtcaaaaattgacgatacctctgcagaattacttacagatgatatatctgatttaaaaaataacaatgatattacagctgaaaacaataatatatataaagcagcaaaagatgtaaccacttccctatcaaaagtattaaagaatatcaataaggattaa

SEQ ID NO: 8 - DNA, 57 bp, Shigella flexneri
  IpaA VBS1
atatataaagcagcaaaagatgtaaccacttccctatcaaaagtattaaagaatatc

SEQ ID NO: 9 - DNA, 57 bp, Shigella flexneri
  IpaA VBS2
atctatgaaaaggcaaaagaagtatctagcgccctcagcaaggtattgtcaaaaatt

SEQ ID NO: 10 - DNA, 57 bp, Shigella flexneri
  IpaA VBS3
atatttgaagcttcaaaaaaagtaacaaactccctaagtaatcttatatctctcatt

SEQ ID NO: 11 - protein, 258 aa, Homo sapiens
  Vinculin domain D1 (HVD1)
MPVFHTRTIESILEPVAQQISHLVIMHEEGEVDGKAIPDLTAPVAAVQAAVSNLVRVGKETVQTTEDQILKRDMPPAFIKVENACTKLVQAAQMLQSDPYSVPARDYLIDGSRGILSGTSDLLLTFDEAEVRKIIRVCKGILEYLTVAEVVETMEDLVTYTKNLGPGMTKMAKMIDERQQELTHQEHRVMLVNSMNTVKELLPVLISAMKIFVTTKNSKNQGIEEALKNRNFTVEKMSAEINEIIRVLQLTSWDEDAW

SEQ ID NO: 12 - protein, 226 aa, Homo sapiens
  Vinculin domain D2 (HVD2)
ASKDTEAMKRALASIDSKLNQAKGWLRDPSASPGDAGEQAIRQILDEAGKVGELCAGKERREILGTCKMLGQMTDQVADLRARGQGSSPVAMQKAQQVSQGLDVLTAKVENAARKLEAMTNSKQSIAKKIDAAQNWLADPNGGPEGEEQIRGALAEARKIAELCDDPKERDDILRSLGEISALTSKLADLRRQGKGDSPEARALAKQVATALQNLQTKTNRAVANS

SEQ ID NO: 13 - protein, 232 aa, Homo sapiens
  Vinculin domain D3 (HVD3)
RPAKAAVHLEGKIEQAQRWIDNPTVDDRGVGQAAIRGLVAEGHRLANVMMGPYRQDLLAKCDRVDQLTAQLADLAARGEGESPQARALASQLQDSLKDLKARMQEAMTQEVSDVFSDTTTPIKLLAVAATAPPDAPNREEVFDERAANFENHSGKLGATAEKAAAVGTANKSTVEGIQASVKTARELTPQVVSAARILLRNPGNQAAYEHFETMKNQWIDNVEKMTGLVDEA

SEQ ID NO: 14 - protein, 118 aa, Homo sapiens
  Vinculin domain D4 (HVD4)
IDTKSLLDASEEAIKKDLDKCKVAMANIQPQMLVAGATSIARRANRILLVAKREVENSEDPKFREAVKAASDELSKTISPMVMDAKAVAGNISDPGLQKSFLDSGYRILGAVAKVREA

SEQ ID NO: 15 - protein, 110 aa, Shigella flexneri
  A524 / IpaA (524-633)
KSKDITKSTTEHRINNKLKVTDANIRNYVTETNADTIDKNHAIYEKAKEVSSALSKVLSKIDDTSAELLTDDISDLKNNNDITAENNNIYKAAKDVTTSLSKVLKNINKD

SEQ ID NO: 16 - DNA, 3201 bp, Artificial Sequence
  Human vinculin construct (HV)
atgccagtgtttcatacgcgcacgatcgagagcatcctggagccggtggcacagcagatctcccacctggtgataatgcacgaggagggcgaggtggacggcaaagccattcctgacctcaccgcgcccgtggccgccgtgcaggcggccgtcagcaacctcgtccgggttggaaaagagactgttcaaaccactgaggatcagattttgaagagagatatgccaccagcatttattaaggttgagaatgcttgcaccaagcttgtccaggcagctcagatgcttcagtcagacccttactcagtgcctgctcgagattatctaattgatgggtcaaggggcatcctctctggaacatcagacctgctccttaccttcgatgaggctgaggtccgtaaaattattagagtttgcaaaggaattttggaatatcttacagtggcagaggtggtggagactatggaagatttggtcacttacacaaagaatcttgggccaggaatgactaagatggccaagatgattgacgagagacagcaggagctcactcaccaggagcaccgagtgatgttggtgaactcgatgaacaccgtgaaagagttgctgccagttctcatttcagctatgaagatttttgtaacaactaaaaactcaaaaaaccaaggcatagaggaagctttaaaaaatcgcaattttactgtagaaaaaatgagtgctgaaattaatgagataattcgtgtgttacaactcacctcttgggatgaagatgcctgggccagcaaggacactgaagccatgaagagagcattggcctccatagactccaaactgaaccaggccaaaggttggctccgtgaccctagtgcctccccaggggatgctggtgagcaggccatcagacagatcttagatgaagctggaaaagttggtgaactctgtgcaggcaaagaacgcagggagattctgggaacttgcaaaatgctagggcagatgactgatcaagtggctgacctccgtgccagaggacaaggatcctcaccggtggccatgcagaaagctcagcaggtatctcagggtctggatgtgctcacagcaaaagtggaaaatgcagctcgcaagctggaagccatgaccaactcaaagcagagcattgcaaagaagatcgatgctgctcagaactggcttgcagatccaaatggtggaccggaaggagaagagcagattcgaggtgctttggctgaagctcggaaaatagcagaattatgtgatgatcctaaagaaagagatgacattctacgttcccttggggaaatatctgctctgacttctaaattagcagatctacgaagacaggggaaaggagattctccagaggctcgagccttggccaaacaggtggccacggccctgcagaacctgcagaccaaaaccaaccgggctgtggccaacagcagaccggccaaagcagctgtacaccttgagggcaagattgagcaagcacagcggtggattgataatcccacagtggatgaccgtggagtcggtcaggctgccatccgggggcttgtggccgaagggcatcgtctggctaatgttatgatggggccttatcggcaagatcttctcgccaagtgtgaccgagtggaccagctgacagcccagctggctgacctggctgccagaggggaaggggagagtcctcaggcacgagcacttgcatctcagctccaagactccttaaaggatctaaaagctcggatgcaggaggccatgactcaggaagtgtcagatgttttcagcgataccacaactcccatcaagctgttggcagtggcagccacggcgcctcctgatgcgcctaacagggaagaggtatttgatgagagggcagctaactttgaaaaccattcaggaaagcttggtgctacggccgagaaggcggctgcggttggtactgctaataaatcaacagtggaaggcattcaggcctcagtgaagacggcccgagaactcacaccccaggtggtctcggctgctcgtatcttacttaggaaccctggaaatcaagctgcttatgaacattttgagaccatgaagaaccagtggatcgataatgttgaaaaaatgacagggctggtggacgaagccattgataccaaatctctgttggatgcttcagaagaagcaattaaaaaagacctggacaagtgcaaggtagctatggccaacattcagcctcagatgctggttgctggggcaaccagtattgctcgtcgggccaaccggatcctgctggtggctaagagggaggtggagaattccgaggatcccaagttccgtgaggctgtgaaagctgcctctgatgaattgagcaaaaccatctccccaatggtgatggatgcaaaagctgtggctggaaacatttccgaccctggactgcaaaagagcttcctggactcaggatatcggatcctgggagctgtggccaaggtcagagaagccttccaacctcaggagcctgacttcccgccgcctccaccagaccttgaacaactccgactaacagatgagcttgctcctcccaaaccacctctgcctgaaggtgaggtccctccacctaggcctccaccaccagaggaaaaggatgaagagttccctgagcagaaggccggggaggtgattaaccagccaatgatgatggctgccagacagctccatgatgaagctcgcaaatggtccagcaagggcaatgacatcattgcagcagccaagcgcatggctctgctgatggctgagatgtctcggctggtaagagggggcagtggtaccaagcgggcactcattcagtgtgccaaggacatcgccaaggcctcagatgaggtgactcggttggccaaggaggttgccaagcagtgcacagataaacggattagaaccaacctcttacaggtatgtgagcgaatcccaaccataagcacccagctcaaaatcctgtccacagtgaaggccaccatgctgggccggaccaacatcagtgatgaggagtctgagcaggccacagagatgctggttcacaatgcccagaacctcatgcagtctgtgaaggagactgtgcgggaagctgaagctgcttcaatcaaaattcgaacagatgctggatttacactgcgctgggttagaaagactccctggtaccagtag

SEQ ID NO: 17 - DNA, 24 bp, Artificial Sequence
  HV Fwd primer
gcgcatatgccagtgtttcatacg

SEQ ID NO: 18 - DNA, 25 bp, Artificial Sequence
  HV Rv primer
cgtcgactcaccaggcatcttcatc

SEQ ID NO: 19 - DNA, 26 bp, Artificial Sequence
  HV Rv primer
cgtcgactcagtgtacagctgctttg

SEQ ID NO: 20 - DNA, 41 bp, Artificial Sequence
  HV_K276R Fwd primer
gcattggcctccatagactcccgtctgaaccaggccaaagg

SEQ ID NO: 21 - DNA, 41 bp, Artificial Sequence
  HV_K276R Rv primer
cctttggcctggttcagacgggagtctatggaggccaatgc

SEQ ID NO: 22 - DNA, 41 bp, Artificial Sequence
  HV_E305Q Fwd primer
ggccatcagacagatcttagatcaagctggaaaagttggtg

SEQ ID NO: 23 - DNA, 41 bp, Artificial Sequence
  HV_E305Q Rv primer
caccaacttttccagcttgatctaagatctgtctgatggcc

SEQ ID NO: 24 - DNA, 22 bp, Artificial Sequence
  GFP-IpaA483 Fwd primer
gcgatatcatggccagcaaagg

SEQ ID NO: 25 - DNA, 29 bp, Artificial Sequence
  GFP-IpaA483 Rv primer
gcgcggccgcttaatccttattgatattc

SEQ ID NO: 26 - DNA, 31 bp, Artificial Sequence
  GST-IpaA483 Fwd primer
ggcgaattcccggagacacatatttaacacg

SEQ ID NO: 27 - DNA, 29 bp, Artificial Sequence
  GST-IpaA483 Rv primer
gccgtcgacttaatccttattgatattct

SEQ ID NO: 28 - DNA, 1242 bp, Artificial Sequence
  GFP-IpaA483
atggccagcaaaggagaagaacttttcactggagttgtcccaattcttgttgaattagatggtgatgttaatgggcacaaattttctgtcagtggagagggtgaaggtgatgctacatacggaaagcttacccttaaatttatttgcactactggaaaactacctgttccatggccaacacttgtcactactttctcttatggtgttcaatgcttttcccgttatccggatcatatgaaacggcatgactttttcaagagtgccatgcccgaaggttatgtacaggaacgcactatatctttcaaagatgacgggaactacaagacgcgtgctgaagtcaagtttgaaggtgatacccttgttaatcgtatcgagttaaaaggtattgattttaaagaagatggaaacattctcggacacaaactcgagtacaactataactcacacaatgtatacatcacggcagacaaacaaaagaatggaatcaaagctaacttcaaaattcgccacaacattgaagatggatccgttcaactagcagaccattatcaacaaaatactccaattggcgatggccctgtccttttaccagacaaccattacctgtcgacacaatctgccctttcgaaagatcccaacgaaaagcgtgaccacatggtccttcttgagtttgtaactgctgctgggattacacatggcatggatgagctctacaaaagcggttccggaccggtgctagcggtaccgagctcggatccactagtccagtgtggtggaattgcccttggagacacatatttaacacgggaaacgatatttgaagcttcaaaaaaagtaacaaactccctaagtaatcttatatctctcattggaactaaatcaggaacacaagaacgagagttacaggaaaaatcaaaggacattacaaaatccacaacagaacatagaataaacaacaaattaaaagttacagatgcaaatataagaaactacgtaacagaaaccaacgcagatacaattgataaaaatcatgcgatctatgaaaaggcaaaagaagtatctagcgccctcagcaaggtattgtcaaaaattgacgatacctctgcagaattacttacagatgatatatctgatttaaaaaataacaatgatattacagctgaaaacaataatatatataaagcagcaaaagatgtaaccacttccctatcaaaagtattaaagaatatcaataaggattaa

SEQ ID NO: 29 - DNA, 1146 bp, Artificial Sequence
  GST-IpaA483
atgtcccctatactaggttattggaaaattaagggccttgtgcaacccactcgacttcttttggaatatcttgaagaaaaatatgaagagcatttgtatgagcgcgatgaaggtgataaatggcgaaacaaaaagtttgaattgggtttggagtttcccaatcttccttattatattgatggtgatgttaaattaacacagtctatggccatcatacgttatatagctgacaagcacaacatgttgggtggttgtccaaaagagcgtgcagagatttcaatgcttgaaggagcggttttggatattagatacggtgtttcgagaattgcatatagtaaagactttgaaactctcaaagttgattttcttagcaagctacctgaaatgctgaaaatgttcgaagatcgtttatgtcataaaacatatttaaatggtgatcatgtaacccatcctgacttcatgttgtatgacgctcttgatgttgttttatacatggacccaatgtgcctggatgcgttcccaaaattagtttgttttaaaaaacgtattgaagctatcccacaaattgataagtacttgaaatccagcaagtatatagcatggcctttgcagggctggcaagccacgtttggtggtggcgaccatcctccaaaatcggatctggttccgcgtggatccccaggaattcccggagacacatatttaacacgggaaacgatatttgaagcttcaaaaaaagtaacaaactccctaagtaatcttatatctctcattggaactaaatcaggaacacaagaacgagagttacaggaaaaatcaaaggacattacaaaatccacaacagaacatagaataaacaacaaattaaaagttacagatgcaaatataagaaactacgtaacagaaaccaacgcagatacaattgataaaaatcatgcgatctatgaaaaggcaaaagaagtatctagcgccctcagcaaggtattgtcaaaaattgacgatacctctgcagaattacttacagatgatatatctgatttaaaaaataacaatgatattacagctgaaaacaataatatatataaagcagcaaaagatgtaaccacttccctatcaaaagtattaaagaatatcaataaggattaa

SEQ ID NO: 30 - RNA, 25 nt, Artificial Sequence
  anti-talin 1 siRNA
ccaagaacggaaaccugccagaguu

SEQ ID NO: 31 - protein, 1066 aa, Homo sapiens
  Human vinculin (HV)
MPVFHTRTIESILEPVAQQISHLVIMHEEGEVDGKAIPDLTAPVAAVQAAVSNLVRVGKETVQTTEDQILKRDMPPAFIKVENACTKLVQAAQMLQSDPYSVPARDYLIDGSRGILSGTSDLLLTFDEAEVRKIIRVCKGILEYLTVAEVVETMEDLVTYTKNLGPGMTKMAKMIDERQQELTHQEHRVMLVNSMNTVKELLPVLISAMKIFVTTKNSKNQGIEEALKNRNFTVEKMSAEINEIIRVLQLTSWDEDAWASKDTEAMKRALASIDSKLNQAKGWLRDPSASPGDAGEQAIRQILDEAGKVGELCAGKERREILGTCKMLGQMTDQVADLRARGQGSSPVAMQKAQQVSQGLDVLTAKVENAARKLEAMTNSKQSIAKKIDAAQNWLADPNGGPEGEEQIRGALAEARKIAELCDDPKERDDILRSLGEISALTSKLADLRRQGKGDSPEARALAKQVATALQNLQTKTNRAVANSRPAKAAVHLEGKIEQAQRWIDNPTVDDRGVGQAAIRGLVAEGHRLANVMMGPYRQDLLAKCDRVDQLTAQLADLAARGEGESPQARALASQLQDSLKDLKARMQEAMTQEVSDVFSDTTTPIKLLAVAATAPPDAPNREEVFDERAANFENHSGKLGATAEKAAAVGTANKSTVEGIQASVKTARELTPQVVSAARILLRNPGNQAAYEHFETMKNQWIDNVEKMTGLVDEAIDTKSLLDASEEAIKKDLDKCKVAMANIQPQMLVAGATSIARRANRILLVAKREVENSEDPKFREAVKAASDELSKTISPMVMDAKAVAGNISDPGLQKSFLDSGYRILGAVAKVREAFQPQEPDFPPPPPDLEQLRLTDELAPPKPPLPEGEVPPPRPPPPEEKDEEFPEQKAGEVINQPMMMAARQLHDEARKWSSKGNDIIAAAKRMALLMAEMSRLVRGGSGTKRALIQCAKDIAKASDEVTRLAKEVAKQCTDKRIRTNLLQVCERIPTISTQLKILSTVKATMLGRTNISDEESEQATEMLVHNAQNLMQSVKETVREAEAASIKIRTDAGFTLRWVRKTPWYQ

SEQ ID NO: 32 - DNA, 333 bp, Shigella flexneri
  A524 / IpaA (524-633)
aaatcaaaggacattacaaaatccacaacagaacatagaataaacaacaaattaaaagttacagatgcaaatataagaaactacgtaacagaaaccaacgcagatacaattgataaaaatcatgcgatctatgaaaaggcaaaagaagtatctagcgccctcagcaaggtattgtcaaaaattgacgatacctctgcagaattacttacagatgatatatctgatttaaaaaataacaatgatattacagctgaaaacaataatatatataaagcagcaaaagatgtaaccacttccctatcaaaagtattaaagaatatcaataaggattaa

SEQ ID NO: 33 - DNA, 837 bp, Artificial Sequence
  Vinculin domain D1 (HVD1)
atgggcagcagccatcatcatcatcatcacagcagcggcctggtgccgcgcggcagccatatgccagtgtttcatacgcgcacgatcgagagcatcctggagccggtggcacagcagatctcccacctggtgataatgcacgaggagggcgaggtggacggcaaagccattcctgacctcaccgcgcccgtggccgccgtgcaggcggccgtcagcaacctcgtccgggttggaaaagagactgttcaaaccactgaggatcagattttgaagagagatatgccaccagcatttattaaggttgagaatgcttgcaccaagcttgtccaggcagctcagatgcttcagtcagacccttactcagtgcctgctcgagattatctaattgatgggtcaaggggcatcctctctggaacatcagacctgctccttaccttcgatgaggctgaggtccgtaaaattattagagtttgcaaaggaattttggaatatcttacagtggcagaggtggtggagactatggaagatttggtcacttacacaaagaatcttgggccaggaatgactaagatggccaagatgattgacgagagacagcaggagctcactcaccaggagcaccgagtgatgttggtgaactcgatgaacaccgtgaaagagttgctgccagttctcatttcagctatgaagatttttgtaacaactaaaaactcaaaaaaccaaggcatagaggaagctttaaaaaatcgcaattttactgtagaaaaaatgagtgctgaaattaatgagataattcgtgtgttacaactcacctcttgggatgaagatgcctggtga

SEQ ID NO: 34 - DNA, 1539 bp, Artificial Sequence
  Vinculin domains D1-D2 (HVD1D2)
atgggcagcagccatcatcatcatcatcacagcagcggcctggtgccgcgcggcagccatatgccagtgtttcatacgcgcacgatcgagagcatcctggagccggtggcacagcagatctcccacctggtgataatgcacgaggagggcgaggtggacggcaaagccattcctgacctcaccgcgcccgtggccgccgtgcaggcggccgtcagcaacctcgtccgggttggaaaagagactgttcaaaccactgaggatcagattttgaagagagatatgccaccagcatttattaaggttgagaatgcttgcaccaagcttgtccaggcagctcagatgcttcagtcagacccttactcagtgcctgctcgagattatctaattgatgggtcaaggggcatcctctctggaacatcagacctgctccttaccttcgatgaggctgaggtccgtaaaattattagagtttgcaaaggaattttggaatatcttacagtggcagaggtggtggagactatggaagatttggtcacttacacaaagaatcttgggccaggaatgactaagatggccaagatgattgacgagagacagcaggagctcactcaccaggagcaccgagtgatgttggtgaactcgatgaacaccgtgaaagagttgctgccagttctcatttcagctatgaagatttttgtaacaactaaaaactcaaaaaaccaaggcatagaggaagctttaaaaaatcgcaattttactgtagaaaaaatgagtgctgaaattaatgagataattcgtgtgttacaactcacctcttgggatgaagatgcctgggccagcaaggacactgaagccatgaagagagcattggcctccatagactccaaactgaaccaggccaaaggttggctccgtgaccctagtgcctccccaggggatgctggtgagcaggccatcagacagatcttagatgaagctggaaaagttggtgaactctgtgcaggcaaagaacgcagggagattctgggaacttgcaaaatgctagggcagatgactgatcaagtggctgacctccgtgccagaggacaaggatcctcaccggtggccatgcagaaagctcagcaggtatctcagggtctggatgtgctcacagcaaaagtggaaaatgcagctcgcaagctggaagccatgaccaactcaaagcagagcattgcaaagaagatcgatgctgctcagaactggcttgcagatccaaatggtggaccggaaggagaagagcagattcgaggtgctttggctgaagctcggaaaatagcagaattatgtgatgatcctaaagaaagagatgacattctacgttcccttggggaaatatctgctctgacttctaaattagcagatctacgaagacaggggaaaggagattctccagaggctcgagccttggccaaacaggtggccacggccctgcagaacctgcagaccaaaaccaaccgggctgtggccaacagcagaccggccaaagcagctgtacactga

SEQ ID NO: 35 - protein, 512 aa, Artificial Sequence
  Vinculin domains D1-D2 (HVD1D2)
MGSSHHHHHHSSGLVPRGSHMPVFHTRTIESILEPVAQQISHLVIMHEEGEVDGKAIPDLTAPVAAVQAAVSNLVRVGKETVQTTEDQILKRDMPPAFIKVENACTKLVQAAQMLQSDPYSVPARDYLIDGSRGILSGTSDLLLTFDEAEVRKIIRVCKGILEYLTVAEVVETMEDLVTYTKNLGPGMTKMAKMIDERQQELTHQEHRVMLVNSMNTVKELLPVLISAMKIFVTTKNSKNQGIEEALKNRNFTVEKMSAEINEIIRVLQLTSWDEDAWASKDTEAMKRALASIDSKLNQAKGWLRDPSASPGDAGEQAIRQILDEAGKVGELCAGKERREILGTCKMLGQMTDQVADLRARGQGSSPVAMQKAQQVSQGLDVLTAKVENAARKLEAMTNSKQSIAKKIDAAQNWLADPNGGPEGEEQIRGALAEARKIAELCDDPKERDDILRSLGEISALTSKLADLRRQGKGDSPEARALAKQVATALQNLQTKTNRAVANSRPAKAAVH

SEQ ID NO: 36 - protein, 512 aa, Artificial Sequence
  Vinculin domains D1-D2 (HVD1D2) K276R
MGSSHHHHHHSSGLVPRGSHMPVFHTRTIESILEPVAQQISHLVIMHEEGEVDGKAIPDLTAPVAAVQAAVSNLVRVGKETVQTTEDQILKRDMPPAFIKVENACTKLVQAAQMLQSDPYSVPARDYLIDGSRGILSGTSDLLLTFDEAEVRKIIRVCKGILEYLTVAEVVETMEDLVTYTKNLGPGMTKMAKMIDERQQELTHQEHRVMLVNSMNTVKELLPVLISAMKIFVTTKNSKNQGIEEALKNRNFTVEKMSAEINEIIRVLQLTSWDEDAWASKDTEAMKRALASIDSRLNQAKGWLRDPSASPGDAGEQAIRQILDEAGKVGELCAGKERREILGTCKMLGQMTDQVADLRARGQGSSPVAMQKAQQVSQGLDVLTAKVENAARKLEAMTNSKQSIAKKIDAAQNWLADPNGGPEGEEQIRGALAEARKIAELCDDPKERDDILRSLGEISALTSKLADLRRQGKGDSPEARALAKQVATALQNLQTKTNRAVANSRPAKAAVH

SEQ ID NO: 37 - protein, 512 aa, Artificial Sequence
  Vinculin domains D1-D2 (HVD1D2) E305Q
MGSSHHHHHHSSGLVPRGSHMPVFHTRTIESILEPVAQQISHLVIMHEEGEVDGKAIPDLTAPVAAVQAAVSNLVRVGKETVQTTEDQILKRDMPPAFIKVENACTKLVQAAQMLQSDPYSVPARDYLIDGSRGILSGTSDLLLTFDEAEVRKIIRVCKGILEYLTVAEVVETMEDLVTYTKNLGPGMTKMAKMIDERQQELTHQEHRVMLVNSMNTVKELLPVLISAMKIFVTTKNSKNQGIEEALKNRNFTVEKMSAEINEIIRVLQLTSWDEDAWASKDTEAMKRALASIDSKLNQAKGWLRDPSASPGDAGEQAIRQILDQAGKVGELCAGKERREILGTCKMLGQMTDQVADLRARGQGSSPVAMQKAQQVSQGLDVLTAKVENAARKLEAMTNSKQSIAKKIDAAQNWLADPNGGPEGEEQIRGALAEARKIAELCDDPKERDDILRSLGEISALTSKLADLRRQGKGDSPEARALAKQVATALQNLQTKTNRAVANSRPAKAAVH

SEQ ID NO: 38 - protein, 155 aa, Homo sapiens
  Talin-1 VBS1 (482-636)
RGHMPPLTSAQQALTGTINSSMQAVQAAQATLDDFDTLPPLGQDAASKAWRKNKMDESKHEIHSQVDAITAGTASVVNLTAGDPAETDYTAVGCAVTTISSNLTEMSRGVKLLAALLEDEGGSGRPLLQAAKGLAGAVSELLRSAQPASAEPRQN

SEQ ID NO: 39 - protein, 26 aa, Homo sapiens
  Talin-1 VBS2 (1944-1969)
AYTKKELIECARRVSEKVSHVLAALQ

SEQ ID NO: 40 - protein, 9 aa, Shigella flexneri
  N-ter Domain
GDTYLTRET

SEQ ID NO: 41 - protein, 55 aa, Shigella flexneri
  Interdomain VBS3-VBS2
GTKSGTQERELQEKSKDITKSTTEHRINNKLKVTDANIRNYVTETNADTIDKNHA

SEQ ID NO: 42 - protein, 27 aa, Shigella flexneri
  Interdomain VBS2-VBS1
DDTSAELLTDDISDLKNNNDITAENNN

SEQ ID NO: 43 - protein, 481 aa, Shigella sonnei
  SipA
NIEHRLALLAQQHTSGEALSLGQKLLNTEVSSFIKNNILAELKLSNETVSSLKLDDLVDAQAKLAFDSLRNQRKNTIDSKGFGIGKLSRDLNTVAVFPELLRKVLNDILEDIKDSHPIQDGLPTPPEDMPDGGPTPGANEKTSQPVIHYHINNDNRTYDNRVFDNRVYDNSYHENPENDAQSPTSQTNDLLSRNGNSLLNPQRALVQKVTSVLPHSISDTVQTFANNSALEKVFNHTPDNSDGIGSDLLTTSSQERSANNSLSRGHRPLNIQNSSTTPPLHPEGVTSSNDNSSDTTKSSASLSHRVASQINKFNSNTDSKVLQTDFFSRNGDTYLTRETIFEASKKVTNSLSNLISLIGTKSGTQERELQEKSKDITKSTTEHRINNKLKVTDANTINYVTETNADTIDKNHAIYEKAKEVSSALSKVLSKIDDTSAELLTDDISDLKNNNDITAENNNIYKAAKDVTTSLSKVLKNINKD

SEQ ID NO: 44 - protein, 500 aa, Shigella sonnei
  SipA
VAQYSELIIKDKLSQDSAFGPWSAKNKKLHQLRQNIEHRLALLAQQHTSGEALSLGQKLLNTEVSSFIKNNILAELKLSNETVSSLKLDDLVDAQAKLAFDSLRNQRKNTIDSKGFGIGKLSRDLNTVAVFPELLRKVLNDILEDIKDSHPIQDGLPTPPEDMPDGGPTPGANEKTSQPVIHYHINNDNRTYDNRVFDNRVYDNSYHENPENDAQSPTSQTNDLLSRNGNSLLNPQRALVQKVTSVLPHSISDTVQTFANNSALEKVFNHTPDNSDGIGSDLLTTSSQERSANNSLSRGHRPLNIQNSSTTPPLHPEGVTSSNDNSSDTTKSSASLSHRVASQINKFNSNTDSKVLQTDFFSRNGDTYLTRETIFEASKKVTNSLSNLISLIGTKSGTQERELQEKSKDITKSTTEHRINNKLKVTDANTINYVTETNADTIDKNHAIYEKAKEVSSALSKVLSKIDDTSAELLTDDISDLKNNNDITAENNNIYKAAKD

SEQ ID NO: 45 - protein, 587 aa, Shigella sonnei 53G
  YopE
MSEKESFATSFNQKCLDFLFSSSGKEDVLRSIYSNSMNAYAKSEILEFSNVLYSLVHQNGLNFENEKGLQKIVAQYSELIIKDKLSQDSAFGPWSAKNKKLHQLRQNIEHRLALLAQQHTSGEALSLGQKLLNTEVSSFIKNNILAELKLSNETVSSLKLDDLVDAQAKLAFDSLRNQRKNTIDSKGFGIGKLSRDLNTVAVFPELLRKVLNDILEDIKDSHPIQDGLPTPPEDMPDGGPTPGANEKTSQPVIHYHINNDNRTYDNRVFDNRVYDNSYHENPENDAQSPTSQTNDLLSRNGNSLLNPQRALVQKVTSVLPHSISDTVQTFANNSALEKVFNHTPDNSDGIGSDLLTTSSQERSANNSLSRGHRPLNIQNSSTTPPLHPEGVTSSNDNSSDTTKSSASLSHRVASQINKFNSNTDSKVLQTDFFSRNGDTYLTRETIFEASKKVTNSLSNLISLIGTKSGTQERELQEKSKDITKSTTEHRINNKLKVTDANTINYVTETNADTIDKNHAIYEKAKEVSSALSKVLSKIDDTSAELLTDDISDLKNNNDITAENNNIYKAAKDVTTSLSKVLKNINKD

SEQ ID NO: 46 - DNA, 1902 bp, Shigella flexneri 6
  pINV_F6_M1382 (3109-5010)
ttaatccttattgatattctttaatacttttgatagggaagtggttacatcttttgctgctttatatatattattgttttcagctgtaatatcattgttattttttaaatcagatatatcatctgtaagtaattctgcagaggtatcgtcaatttttgacaataccttgctgagggcgctagatacttcttttgccttttcatagatcgcatgatttttatcaattgtatctgcgttggtttctgttacgtagtttattgtatttgcatctgtaacttttaatttgttgtttattctgtgttctgttgtggattttgtaatgtcctttgatttttcctgtaactctcgttcttgtgttcctgatttagttccaatgagagatataagattacttagggagtttgttactttttttgaagcttcaaatatcgtttcccgtgttaaatatgtgtctccatttcttgataaaaaatcagtctgaagtacttttgaatcagtgtttgagttgaatttattgatttgcgaagctactctatgagaaagagaagcgctacttttagttgtatctgatgagttatcattactgcttgtcactccttccgggtggagagggggggtggttgaagagttctgtatgttcagaggcctgtgtccccgagaaagagagttatttgtagatctttcttgactactcgtagttaacaggtctgaacctattccatccgaattatctggagtatggttgaaaaccttttctaaagctgaattatttgcaaatgtctggacagcatctgatatagagtgtggtagaacggaagttactttttgaactagtgctctttgtggatttagtaatgagtttccgttacgggataatagatcgtttgtctgagaagtaggagactgtgcatcattttctgggttctcgtgatagctattgtcatatactctgttgtcaaaaactctattatcgtaagttctattatcattatttatatgatagtgaattacaggttgggatgttttctcattggctccgggggttggtccgccatctggcatatcttcgggaggtgtagggaggccatcttggataggatgcgaatcttttatatcttctaaaatatcattaaggacttttctcaacagctcaggaaacacggctactgtatttaagtctcttgacagtttacctataccaaatcctttactatcaatagtatttttacgttgattgcgcaaactatcaaaggcaagttttgcctgtgcgtcaactaaatcatctagtttgagagatgaaacagtttcattacttaactttaattcagcaagaatattattcttgataaatgatgatacttcagtattgaggagtttttgtcccaatgataaagcttcaccagatgtgtgttgttgtgctaatagtgcaagtctgtgctcaatgttttgtcgtaattgatggagtttcttattctttgccgaccatggtccaaaggcagaatcttgggataatttatcttttataattagttccgaatactgtgcgacaattttttgaagtcccttttcgttttcaaaattaagatcattttgatgtactaaggagtacaaaacatttgaaaattcgagaatctcgcttttggcatacgcattcattgagttggaataaatgcttcttaacacatcttctttccctgaggaagaaaataaaaaatcaagacatttctgattaaaagacgttgcaaagttttctttttcagacactgatgctggtgtttttagagaagtttgcgaactatggatatcggatattttgctttttaactcgctgtattctgttgatgatggtgaagttgccttatataagaatgttggcgcttgagtattatttacattatgcat

SEQ ID NO: 47 - protein, 20 aa, Chlamydia trachomatis L2
  TarP VBS1
LFQAATQTTQALSSLIDTVG

SEQ ID NO: 48 - protein, 24 aa, Chlamydia trachomatis L2
  TarP VBS2
LFQAAAVTQALGNVAGKVNLAIQG

SEQ ID NO: 49 - protein, 19 aa, Chlamydophila caviae GPIC
  TarP VBS1
LLEAARNTTTMLSKTLSKV

SEQ ID NO: 50 - protein, 19 aa, Chlamydophila caviae GPIC
  TarP VBS2
IPGAAANVTATLSSVANKI

SEQ ID NO: 51 - protein, 19 aa, Chlamydophila caviae GPIC
  TarP VBS3
LHGAAKGVADSLSNLLQAA

SEQ ID NO: 52 - protein, 19 aa, Chlamydophila abortus
  TarP VBS1
LADAARNVTTQLSKTLSKA

SEQ ID NO: 53 - protein, 19 aa, Chlamydophila abortus
  TarP VBS2
IPEAAGNVIQALSNVAKKI

SEQ ID NO: 54 - protein, 19 aa, Chlamydophila abortus
  TarP VBS3
LHGAARDVASSLSNLLEAA

SEQ ID NO: 55 - protein, 19 aa, Chlamydophila felis
  TarP VBS1
LFDAAKQTTAQLSKMIYRA

SEQ ID NO: 56 - protein, 19 aa, Chlamydophila felis
  TarP VBS2
IPQAAANVTQTLSNVTQKL

SEQ ID NO: 57 - protein, 19 aa, Chlamydophila felis
  TarP VBS3
LYAAAGNVADSLSNLLQAA

SEQ ID NO: 58 - protein, 19 aa, Chlamydia muridarum
  TarP VBS1
LFAAARATTQSLSSLIGTV

SEQ ID NO: 59 - protein, 19 aa, Chlamydia muridarum
  TarP VBS2
LYDAAKNVTQALTSVTNKV

SEQ ID NO: 60 - protein, 26 aa, Homo sapiens
  Talin-1 Helix 46 (H46)
YTKKELIECARRVSEKVSHVLAALQA

SEQ ID NO: 61 - protein, 9 aa, Shigella flexneri 5a
  N-ter domain
GDPYLTRET

SEQ ID NO: 62 - protein, 55 aa, Shigella flexneri 5a
  Interdomain VBS3-VBS2
GTKSGTQERELQEKSKDITKSTTEHRINNKLKITDANTINYVTETNADTIDKNHA

SEQ ID NO: 63 - protein, 55 aa, Shigella sonnei 53G
  Interdomain VBS3-VBS2
GTKSGTQERELQEKSKDITKSTTEHRINNKLKVTDANTINYVTETNADTIDKNHA

SEQ ID NO: 64 - protein, 55 aa, Shigella dysenteriae
  Interdomain VBS3-VBS2
GTKSGTQERELQEKSKDITKSTTEHRINNKLKITDANTRNYVTETNADTIDKNHA

SEQ ID NO: 65 - protein, 27 aa, Shigella flexneri 5a
  Interdomain VBS2-VBS1
DDTSAELLTEDISNLKNNNDITAENNN

SEQ ID NO: 66 - protein, 22 aa, Shigella flexneri
  IpaA VBS1
IYKAAKDVTTSLSKVLKNINKD

SEQ ID NO: 67 - protein, 21 aa, Shigella flexneri
  IpaA VBS2
IYEKAKEVSSALSKVLSKIDD

SEQ ID NO: 68 - protein, 25 aa, Shigella flexneri
  IpaA VBS3
TRETIFEASKKVTNSLSNLISLIGT

SEQ ID NO: 69 - DNA, 66 bp, Shigella flexneri
  IpaA VBS1
atatataaagcagcaaaagatgtaaccacttccctatcaaaagtattaaagaatatcaataaggat

SEQ ID NO: 70 - DNA, 63 bp, Shigella flexneri
  IpaA VBS2
atctatgaaaaggcaaaagaagtatctagcgccctcagcaaggtattgtcaaaaattgacgat

SEQ ID NO: 71 - DNA, 75 bp, Shigella flexneri
  IpaA VBS3
acacgggaaacgatatttgaagcttcaaaaaaagtaacaaactccctaagtaatcttatatctctcattggaact

SEQ ID NO: 72 - protein, 5 aa, Shigella flexneri
  N-ter domain
GDTYL

SEQ ID NO: 73 - protein, 53 aa, Shigella flexneri
  Interdomain VBS3-VBS2
KSGTQERELQEKSKDITKSTTEHRINNKLKVTDANIRNYVTETNADTIDKNHA

SEQ ID NO: 74 - protein, 25 aa, Shigella flexneri
  Interdomain VBS2-VBS1
TSAELLTDDISDLKNNNDITAENNN

SEQ ID NO: 75 - protein, 5 aa, Shigella flexneri 5a
  N-ter domain
GDPYL

SEQ ID NO: 76 - protein, 53 aa, Shigella flexneri 5a
  Interdomain VBS3-VBS2
KSGTQERELQEKSKDITKSTTEHRINNKLKITDANTINYVTETNADTIDKNHA

SEQ ID NO: 77 - protein, 53 aa, Shigella sonnei 53G
  Interdomain VBS3-VBS2
KSGTQERELQEKSKDITKSTTEHRINNKLKVTDANTINYVTETNADTIDKNHA

SEQ ID NO: 78 - protein, 53 aa, Shigella dysenteriae
  Interdomain VBS3-VBS2
KSGTQERELQEKSKDITKSTTEHRINNKLKITDANTRNYVTETNADTIDKNHA

SEQ ID NO: 79 - protein, 25 aa, Shigella flexneri 5a
  Interdomain VBS2-VBS1
TSAELLTEDISNLKNNNDITAENNN